European Patent Application EP 4 332 577 A1, published March 6, 2024. Title: APPLICATION OF CRMP2 AND ANTI-CRMP2 ANTIBODIES. Applicant: NANFANG HOSPITAL, SOUTHERN MEDICAL UNIVERSITY. The sequence listing filed with the application follows.

SEQUENCE LISTING (13 sequences)

SEQ ID NO: 1 - protein, 677 aa, Homo sapiens
MAERKQSGKAAEDEEVPAFFKNLGSGSPKPRQKFCGMFCPVEGSSENKTIDFDSLSVGRGSGQVVAQQRDVAHLGPDPQPPYSRQGRRAGGEPSVESGRKVEIRRASGKEALQNINDQSDRLLIKGGKIVNDDQSFYADIYMEDGLIKQIGENLIVPGGVKTIEAHSRMVIPGGIDVHTRFQMPDQGMTSADDFFQGTKAALAGGTTMIIDHVVPEPGTSLLAAFDQWREWADSKSCCDYSLHVDISEWHKGIQEEMEALVKDHGVNSFLVYMAFKDRFQLTDCQIYEVLSVIRDIGAIAQVHAENGDIIAEEQQRILDLGITGPEGHVLSRPEEVEAEAVNRAITIANQTNCPLYITKVMSKSSAEVIAQARKKGTVVYGEPITASLGTDGSHYWSKNWAKAAAFVTSPPLSPDPTTPDFLNSLLSCGDLQVTGSAHCTFNTAQKAVGKDNFTLIPEGTNGTEERMSVIWDKAVVTGKMDENQFVAVTSTNAAKVFNLYPRKGRIAVGSDADLVIWDPDSVKTISAKTHNSSLEYNIFEGMECRGSPLVVISQGKIVLEDGTLHVTEGSGRYIPRKPFPDFVYKRIKARSRLAELRGVPRGLYDGPVCEVSVTPKTVTPASSAKTSPAKQQAPPVRNLHQSGFSLSGAQIDDNIPRRTTQRIVAPPGGRANITSLG

SEQ ID NO: 2 - protein, 572 aa, Homo sapiens
MSYQGKKNIPRITSDRLLIKGGKIVNDDQSFYADIYMEDGLIKQIGENLIVPGGVKTIEAHSRMVIPGGIDVHTRFQMPDQGMTSADDFFQGTKAALAGGTTMIIDHVVPEPGTSLLAAFDQWREWADSKSCCDYSLHVDISEWHKGIQEEMEALVKDHGVNSFLVYMAFKDRFQLTDCQIYEVLSVIRDIGAIAQVHAENGDIIAEEQQRILDLGITGPEGHVLSRPEEVEAEAVNRAITIANQTNCPLYITKVMSKSSAEVIAQARKKGTVVYGEPITASLGTDGSHYWSKNWAKAAAFVTSPPLSPDPTTPDFLNSLLSCGDLQVTGSAHCTFNTAQKAVGKDNFTLIPEGTNGTEERMSVIWDKAVVTGKMDENQFVAVTSTNAAKVFNLYPRKGRIAVGSDADLVIWDPDSVKTISAKTHNSSLEYNIFEGMECRGSPLVVISQGKIVLEDGTLHVTEGSGRYIPRKPFPDFVYKRIKARSRLAELRGVPRGLYDGPVCEVSVTPKTVTPASSAKTSPAKQQAPPVRNLHQSGFSLSGAQIDDNIPRRTTQRIVAPPGGRANITSLG

SEQ ID NO: 3 - protein, 536 aa, Homo sapiens
MEDGLIKQIGENLIVPGGVKTIEAHSRMVIPGGIDVHTRFQMPDQGMTSADDFFQGTKAALAGGTTMIIDHVVPEPGTSLLAAFDQWREWADSKSCCDYSLHVDISEWHKGIQEEMEALVKDHGVNSFLVYMAFKDRFQLTDCQIYEVLSVIRDIGAIAQVHAENGDIIAEEQQRILDLGITGPEGHVLSRPEEVEAEAVNRAITIANQTNCPLYITKVMSKSSAEVIAQARKKGTVVYGEPITASLGTDGSHYWSKNWAKAAAFVTSPPLSPDPTTPDFLNSLLSCGDLQVTGSAHCTFNTAQKAVGKDNFTLIPEGTNGTEERMSVIWDKAVVTGKMDENQFVAVTSTNAAKVFNLYPRKGRIAVGSDADLVIWDPDSVKTISAKTHNSSLEYNIFEGMECRGSPLVVISQGKIVLEDGTLHVTEGSGRYIPRKPFPDFVYKRIKARSRLAELRGVPRGLYDGPVCEVSVTPKTVTPASSAKTSPAKQQAPPVRNLHQSGFSLSGAQIDDNIPRRTTQRIVAPPGGRANITSLG

SEQ ID NO: 4 - DNA, 2034 bp, Homo sapiens
atggccgagagaaagcaatccgggaaggcggcagaggacgaagaggtccctgctttttttaaaaacctgggctccggcagccccaagccccggcagaaattctgtggcatgttctgcccggtggaagggtcctcggagaacaagaccatcgacttcgactcgctgtcggtgggccggggctcggggcaggtggtggctcagcagcgggacgtcgcccacttgggcccggacccgcagccgccgtactcgcggcagggccggcgcgccggcggagagccatctgttgaatcgggccggaaggtggagatccggagggcctcgggcaaagaagccctgcagaacatcaacgaccagagcgatcgtcttctgatcaaaggaggtaaaattgttaatgatgaccagtcgttctatgcagacatatacatggaagatgggttgatcaagcaaataggagaaaatctgattgtgccaggaggagtgaagaccatcgaggcccactcccggatggtgatccccggaggaattgacgtccacactcgtttccagatgcctgatcagggaatgacgtctgctgatgatttcttccaaggaaccaaggcggccctggctgggggaaccactatgatcattgaccacgttgttcctgagcctgggacaagcctgctcgctgcctttgaccagtggagggaatgggccgacagcaagtcctgctgtgactactctctgcatgtggacatcagtgagtggcataagggcatccaggaggagatggaagcgcttgtgaaggatcacggggtaaattccttcctcgtgtacatggctttcaaagatcgcttccagctaacggattgccagatttatgaagtactgagtgtgatccgggatattggcgccatagcccaagtccacgcagaaaatggcgacatcattgcagaggagcagcagaggatcctggatctgggcatcacgggccccgagggacatgtgctgagccgacctgaggaggtcgaggccgaagccgtgaatcgtgccatcaccatcgccaaccagaccaactgcccgctgtatatcaccaaggtgatgagcaaaagctctgctgaggtcatcgcccaggcacggaagaagggaactgtggtgtatggcgagcccatcactgccagcttgggaacggacggctcccattactggagcaagaactgggccaaggctgctgcctttgtcacctccccacccttgagccctgatccaaccactccagactttctcaactccttgctgtcctgtggagacctccaggtcacgggcagtgcccattgcacgtttaacactgcccagaaggctgtaggaaaggacaacttcaccctgattccggagggcaccaatggcactgaggagcggatgtccgtcatctgggacaaggctgtggtcactgggaagatggatgagaaccagtttgtggctgtgaccagcaccaatgcagccaaagtcttcaacctttacccccggaaaggccgcattgctgtgggatccgatgccgacctggtcatctgggaccccgacagcgttaaaaccatctctgccaagacacacaacagctctctcgagtacaacatctttgaaggcatggagtgccgcggctccccactggtggtcatcagccaggggaagattgtcctggaggacggcaccctgcatgtcaccgaaggctctggacgctacattccccggaagcccttccctgattttgtttacaagcgtatcaaggcaaggagcaggctggctgagctgagaggggttcctcgtggcctgtatgacggacctgtgtgtgaagtgtctgtgacgcccaagacagtcactccagcctcctcggccaagacgtctcctgccaagcagcaggccccacctgtccggaacctgcaccagtctggattcagtttgtctggtgctcagattgatgacaacattccccgccgcaccacccagcgtatcgtggcgccccccggtggccgtgccaacatcaccagcctgggctag

SEQ ID NO: 5 - DNA, 1719 bp, Homo sapiens
atgtcttatcaggggaagaaaaatattccacgcatcacgagcgatcgtcttctgatcaaaggaggtaaaattgttaatgatgaccagtcgttctatgcagacatatacatggaagatgggttgatcaagcaaataggagaaaatctgattgtgccaggaggagtgaagaccatcgaggcccactcccggatggtgatccccggaggaattgacgtccacactcgtttccagatgcctgatcagggaatgacgtctgctgatgatttcttccaaggaaccaaggcggccctggctgggggaaccactatgatcattgaccacgttgttcctgagcctgggacaagcctgctcgctgcctttgaccagtggagggaatgggccgacagcaagtcctgctgtgactactctctgcatgtggacatcagtgagtggcataagggcatccaggaggagatggaagcgcttgtgaaggatcacggggtaaattccttcctcgtgtacatggctttcaaagatcgcttccagctaacggattgccagatttatgaagtactgagtgtgatccgggatattggcgccatagcccaagtccacgcagaaaatggcgacatcattgcagaggagcagcagaggatcctggatctgggcatcacgggccccgagggacatgtgctgagccgacctgaggaggtcgaggccgaagccgtgaatcgtgccatcaccatcgccaaccagaccaactgcccgctgtatatcaccaaggtgatgagcaaaagctctgctgaggtcatcgcccaggcacggaagaagggaactgtggtgtatggcgagcccatcactgccagcttgggaacggacggctcccattactggagcaagaactgggccaaggctgctgcctttgtcacctccccacccttgagccctgatccaaccactccagactttctcaactccttgctgtcctgtggagacctccaggtcacgggcagtgcccattgcacgtttaacactgcccagaaggctgtaggaaaggacaacttcaccctgattccggagggcaccaatggcactgaggagcggatgtccgtcatctgggacaaggctgtggtcactgggaagatggatgagaaccagtttgtggctgtgaccagcaccaatgcagccaaagtcttcaacctttacccccggaaaggccgcattgctgtgggatccgatgccgacctggtcatctgggaccccgacagcgttaaaaccatctctgccaagacacacaacagctctctcgagtacaacatctttgaaggcatggagtgccgcggctccccactggtggtcatcagccaggggaagattgtcctggaggacggcaccctgcatgtcaccgaaggctctggacgctacattccccggaagcccttccctgattttgtttacaagcgtatcaaggcaaggagcaggctggctgagctgagaggggttcctcgtggcctgtatgacggacctgtgtgtgaagtgtctgtgacgcccaagacagtcactccagcctcctcggccaagacgtctcctgccaagcagcaggccccacctgtccggaacctgcaccagtctggattcagtttgtctggtgctcagattgatgacaacattccccgccgcaccacccagcgtatcgtggcgccccccggtggccgtgccaacatcaccagcctgggctag

SEQ ID NO: 6 - DNA, 1611 bp, Homo sapiens
atggaagatgggttgatcaagcaaataggagaaaatctgattgtgccaggaggagtgaagaccatcgaggcccactcccggatggtgatccccggaggaattgacgtccacactcgtttccagatgcctgatcagggaatgacgtctgctgatgatttcttccaaggaaccaaggcggccctggctgggggaaccactatgatcattgaccacgttgttcctgagcctgggacaagcctgctcgctgcctttgaccagtggagggaatgggccgacagcaagtcctgctgtgactactctctgcatgtggacatcagtgagtggcataagggcatccaggaggagatggaagcgcttgtgaaggatcacggggtaaattccttcctcgtgtacatggctttcaaagatcgcttccagctaacggattgccagatttatgaagtactgagtgtgatccgggatattggcgccatagcccaagtccacgcagaaaatggcgacatcattgcagaggagcagcagaggatcctggatctgggcatcacgggccccgagggacatgtgctgagccgacctgaggaggtcgaggccgaagccgtgaatcgtgccatcaccatcgccaaccagaccaactgcccgctgtatatcaccaaggtgatgagcaaaagctctgctgaggtcatcgcccaggcacggaagaagggaactgtggtgtatggcgagcccatcactgccagcttgggaacggacggctcccattactggagcaagaactgggccaaggctgctgcctttgtcacctccccacccttgagccctgatccaaccactccagactttctcaactccttgctgtcctgtggagacctccaggtcacgggcagtgcccattgcacgtttaacactgcccagaaggctgtaggaaaggacaacttcaccctgattccggagggcaccaatggcactgaggagcggatgtccgtcatctgggacaaggctgtggtcactgggaagatggatgagaaccagtttgtggctgtgaccagcaccaatgcagccaaagtcttcaacctttacccccggaaaggccgcattgctgtgggatccgatgccgacctggtcatctgggaccccgacagcgttaaaaccatctctgccaagacacacaacagctctctcgagtacaacatctttgaaggcatggagtgccgcggctccccactggtggtcatcagccaggggaagattgtcctggaggacggcaccctgcatgtcaccgaaggctctggacgctacattccccggaagcccttccctgattttgtttacaagcgtatcaaggcaaggagcaggctggctgagctgagaggggttcctcgtggcctgtatgacggacctgtgtgtgaagtgtctgtgacgcccaagacagtcactccagcctcctcggccaagacgtctcctgccaagcagcaggccccacctgtccggaacctgcaccagtctggattcagtttgtctggtgctcagattgatgacaacattccccgccgcaccacccagcgtatcgtggcgccccccggtggccgtgccaacatcaccagcctgggctag

SEQ ID NO: 7 - DNA, 2046 bp, Artificial Sequence
  synthesized
ggatccatggccgagagaaagcaatccgggaaggcggcagaggacgaagaggtccctgctttttttaaaaacctgggctccggcagccccaagccccggcagaaattctgtggcatgttctgcccggtggaagggtcctcggagaacaagaccatcgacttcgactcgctgtcggtgggccggggctcggggcaggtggtggctcagcagcgggacgtcgcccacttgggcccggacccgcagccgccgtactcgcggcagggccggcgcgccggcggagagccatctgttgaatcgggccggaaggtggagatccggagggcctcgggcaaagaagccctgcagaacatcaacgaccagagcgatcgtcttctgatcaaaggaggtaaaattgttaatgatgaccagtcgttctatgcagacatatacatggaagatgggttgatcaagcaaataggagaaaatctgattgtgccaggaggagtgaagaccatcgaggcccactcccggatggtgatccccggaggaattgacgtccacactcgtttccagatgcctgatcagggaatgacgtctgctgatgatttcttccaaggaaccaaggcggccctggctgggggaaccactatgatcattgaccacgttgttcctgagcctgggacaagcctgctcgctgcctttgaccagtggagggaatgggccgacagcaagtcctgctgtgactactctctgcatgtggacatcagtgagtggcataagggcatccaggaggagatggaagcgcttgtgaaggatcacggggtaaattccttcctcgtgtacatggctttcaaagatcgcttccagctaacggattgccagatttatgaagtactgagtgtgatccgggatattggcgccatagcccaagtccacgcagaaaatggcgacatcattgcagaggagcagcagaggatcctggatctgggcatcacgggccccgagggacatgtgctgagccgacctgaggaggtcgaggccgaagccgtgaatcgtgccatcaccatcgccaaccagaccaactgcccgctgtatatcaccaaggtgatgagcaaaagctctgctgaggtcatcgcccaggcacggaagaagggaactgtggtgtatggcgagcccatcactgccagcttgggaacggacggctcccattactggagcaagaactgggccaaggctgctgcctttgtcacctccccacccttgagccctgatccaaccactccagactttctcaactccttgctgtcctgtggagacctccaggtcacgggcagtgcccattgcacgtttaacactgcccagaaggctgtaggaaaggacaacttcaccctgattccggagggcaccaatggcactgaggagcggatgtccgtcatctgggacaaggctgtggtcactgggaagatggatgagaaccagtttgtggctgtgaccagcaccaatgcagccaaagtcttcaacctttacccccggaaaggccgcattgctgtgggatccgatgccgacctggtcatctgggaccccgacagcgttaaaaccatctctgccaagacacacaacagctctctcgagtacaacatctttgaaggcatggagtgccgcggctccccactggtggtcatcagccaggggaagattgtcctggaggacggcaccctgcatgtcaccgaaggctctggacgctacattccccggaagcccttccctgattttgtttacaagcgtatcaaggcaaggagcaggctggctgagctgagaggggttcctcgtggcctgtatgacggacctgtgtgtgaagtgtctgtgacgcccaagacagtcactccagcctcctcggccaagacgtctcctgccaagcagcaggccccacctgtccggaacctgcaccagtctggattcagtttgtctggtgctcagattgatgacaacattccccgccgcaccacccagcgtatcgtggcgccccccggtggccgtgccaacatcaccagcctgggctaggaattc

SEQ ID NO: 8 - protein, 572 aa, Artificial Sequence
  synthesized
  misc_feature (2)..(4): Xaa can be any naturally occurring amino acid
  misc_feature (7)..(11): Xaa can be any naturally occurring amino acid
  misc_feature (13)..(13): Xaa can be any naturally occurring amino acid
MXXXGKXXXXXIXSDRLLIKGGKIVNDDQSFYADIYMEDGLIKQIGENLIVPGGVKTIEAHSRMVIPGGIDVHTRFQMPDQGMTSADDFFQGTKAALAGGTTMIIDHVVPEPGTSLLAAFDQWREWADSKSCCDYSLHVDISEWHKGIQEEMEALVKDHGVNSFLVYMAFKDRFQLTDCQIYEVLSVIRDIGAIAQVHAENGDIIAEEQQRILDLGITGPEGHVLSRPEEVEAEAVNRAITIANQTNCPLYITKVMSKSSAEVIAQARKKGTVVYGEPITASLGTDGSHYWSKNWAKAAAFVTSPPLSPDPTTPDFLNSLLSCGDLQVTGSAHCTFNTAQKAVGKDNFTLIPEGTNGTEERMSVIWDKAVVTGKMDENQFVAVTSTNAAKVFNLYPRKGRIAVGSDADLVIWDPDSVKTISAKTHNSSLEYNIFEGMECRGSPLVVISQGKIVLEDGTLHVTEGSGRYIPRKPFPDFVYKRIKARSRLAELRGVPRGLYDGPVCEVSVTPKTVTPASSAKTSPAKQQAPPVRNLHQSGFSLSGAQIDDNIPRRTTQRIVAPPGGRANITSLG

SEQ ID NO: 9 - protein, 572 aa, Mus musculus
MSYQGKKNIPRITSDRLLIKGGKIVNDDQSFYADIYMEDGLIKQIGENLIVPGGVKTIEAHSRMVIPGGIDVHTRFQMPDQGMTSADDFFQGTKAALAGGTTMIIDHVVPEPGTSLLAAFDQWREWADSKSCCDYSLHVDITEWHKGIQEEMEALVKDHGVNSFLVYMAFKDRFQLTDSQIYEVLSVIRDIGAIAQVHAENGDIIAEEQQRILDLGITGPEGHVLSRPEEVEAEAVNRSITIANQTNCPLYVTKVMSKSAAEVIAQARKKGTVVYGEPITASLGTDGSHYWSKNWAKAAAFVTSPPLSPDPTTPDFLNSLLSCGDLQVTGSAHCTFNTAQKAVGKDNFTLIPEGTNGTEERMSVIWDKAVVTGKMDENQFVAVTSTNAAKVFNLYPRKGRISVGSDADLVIWDPDSVKTISAKTHNSALEYNIFEGMECRGSPLVVISQGKIVLEDGTLHVTEGSGRYIPRKPFPDFVYKRIKARSRLAELRGVPRGLYDGPVCEVSVTPKTVTPASSAKTSPAKQQAPPVRNLHQSGFSLSGAQIDDNIPRRTTQRIVAPPGGRANITSLG

SEQ ID NO: 10 - protein, 572 aa, Rattus norvegicus; identical to SEQ ID NO: 9

SEQ ID NO: 11 - protein, 572 aa, Bos taurus [sequence omitted]

SEQ ID NO: 12 - protein, 572 aa, Pongo pygmaeus; identical to SEQ ID NO: 2

SEQ ID NO: 13 - protein, 572 aa, Gallus gallus
MSYQGKKNIPRITSDRLLIKGGKIVNDDQSFYADIYMEDGLIKQIGENLIVPGGVKTIEAHGRMVIPGGIDVHTRFQMPEQGMTSADDFFQGTKAALAGGTTMIIDHVVPEPGTSLLTAFDQWREWADSKSCCDYSLHVDITEWHKGVQEEMEALVKDHGVNSFLVYMAFKDRFQLSDSQIYEVLSVIRDIGATAQVHAENGDIIAEEQQRILELGITGPEGHVLSRPEEVEAEAVNRAITIANQTNCPLYITKVMSKSAAEVIAQARKKGTVVYGEPITASLGTDGSHYWSKNWAKAAAFVTSPPLSPDPTTPDFLNSLLSCGDLQVTGSAHCTFNTAQKAVGKDNFTLIPEGTNGTEERMSIIWDKAVVTGKMDENQFVAVTSTNAAKIFNLYPRKGRIAVGSDADLVIWDPDSVKTISAKTHNISLEYNIFEGMECRGSPLVVISQGKIVLEDGNLHVTEGSGRYIPRKPFPDFVYKRIKARSRLAELRGVPRGLYDGPVCEVSVTPKTVTPASSAKTSPAKQQAPPVRNLHQSGFSLSGAQIDDNIPRRTTQRIVAPPGGRANITSLG